European Patent Application EP 4 155 409 A1, published March 29, 2023. Title: METHOD OF INCREASING THE REPLICATION OF A CIRCULAR DNA MOLECULE. Applicant: CureVac Real Estate GmbH. Application EP. The sequence listing filed with the application follows.

SEQUENCE LISTING (17 sequences)

SEQ ID NO: 1 - DNA, 100 bp, synthetic construct
  misc_feature 1..100: note = poly(A) and poly(c) sequence
  source 1..100: mol_type = other DNA
aaaaaaaaaaaaaaaaaaaaaaaaaaaaaaaaaaaaaaaaaaaaaaaaaaaaaaaaaaaaaaaatgcatccccccccccccccccccccccccccccccc

SEQ ID NO: 2 - RNA, 2083 nt, synthetic construct
  misc_feature 1..2083: note = GC-optimized mRNA H1N1
  source 1..2083: mol_type = other RNA
ggggcgctgcctacggaggtggcagccatctccttctcggcatcaagcttaccatgaaggccatcctggtggtcctcctgtacaccttcgccaccgcgaacgccgacacgctgtgcatcggctaccacgccaacaacagcaccgacaccgtggacaccgtgctcgagaagaacgtcacggtgacccactccgtgaacctgctggaggacaagcacaacgggaagctctgcaagctgcggggcgtcgccccgctgcacctcgggaagtgcaacatcgccggctggatcctggggaacccggagtgcgagagcctgtccaccgcgagctcctggagctacatcgtggagacctccagctccgacaacggcacgtgctaccccggcgacttcatcgactacgaggagctccgcgagcagctgagctccgtgagctccttcgagcggttcgagatcttccccaagaccagctcctggcccaaccacgacagcaacaagggggtcaccgccgcctgcccgcacgccggcgcgaagtccttctacaagaacctgatctggctcgtgaagaaggggaacagctaccccaagctgtccaagagctacatcaacgacaagggcaaggaggtgctggtcctctgggggatccaccaccccagcacctccgccgaccagcagagcctgtaccagaacgccgacgcctacgtgttcgtgggctccagccgctactccaagaagttcaagcccgagatcgccatccggccgaaggtccgcgaccaggagggccggatgaactactactggacgctggtggagcccggggacaagatcaccttcgaggcgaccggcaacctcgtggtcccccgctacgccttcgccatggagcggaacgccgggagcggcatcatcatctccgacacccccgtgcacgactgcaacacgacctgccagaccccgaagggcgccatcaacaccagcctgcccttccagaacatccaccccatcacgatcgggaagtgccccaagtacgtgaagtccaccaagctgcgcctcgcgaccggcctgcggaacgtcccgagcatccagtcccgcgggctgttcggcgccatcgccgggttcatcgagggcggctggaccgggatggtggacggctggtacgggtaccaccaccagaacgagcagggcagcgggtacgccgccgacctcaagtccacgcagaacgcgatcgacgagatcaccaacaaggtgaacagcgtcatcgagaagatgaacacccagttcaccgccgtgggcaaggagttcaaccacctggagaagcggatcgagaacctgaacaagaaggtcgacgacggcttcctcgacatctggacgtacaacgccgagctgctggtgctcctggagaacgagcgcaccctggactaccacgactccaacgtgaagaacctctacgagaaggtccggagccagctgaagaacaacgccaaggagatcgggaacggctgcttcgagttctaccacaagtgcgacaacacctgcatggagtccgtgaagaacgggacctacgactaccccaagtacagcgaggaggccaagctgaaccgcgaggagatcgacggcgtgaagctcgagtccacgcggatctaccagatcctggcgatctacagcaccgtcgccagctccctggtgctcgtggtcagcctgggggccatctccttctggatgtgcagcaacggctccctgcagtgccgcatctgcatctgaccactagtgcatcacatttaaaagcatctcagcctaccatgagaataagagaaagaaaatgaagatcaatagcttattcatctctttttctttttcgttggtgtaaagccaacaccctgtctaaaaaacataaatttctttaatcattttgcctcttttctctgtgcttcaattaataaaaaatggaaagaacctagatctaaaaaaaaaaaaaaaaaaaaaaaaaaaaaaaaaaaaaaaaaaaaaaaaaaaaaaaaaaaaaaaatgcatcccccccccccccccccccccccccccccccaaaggctcttttcagagccaccagaatt

SEQ ID NO: 3 - DNA, 285 bp, synthetic construct
  misc_feature 1..285: note = PAS-BH
  source 1..285: mol_type = other DNA
ctgcctcgcgcgtttcggtgatgacggtgaaaacctctgacacatgcagctcccggagacggtcacagcttgtctgtaagcggatgccgggagcagacaagcccgtcagggcgcgtcagcgggtgttggcgggtgtcggggcgcagccatgacccagtcacgtagcgatagcggagtgtatactggcttaactatgcggcatcagagcagattgtactgagagtgcaccatatgcggtgtgaaataccgcacagatgcgtaaggagaaaataccgcatcaggcgc

SEQ ID NO: 4 - DNA, 1520 bp, synthetic construct
  misc_feature 1..1520: note = P1140-AF-backbone
  source 1..1520: mol_type = other DNA
ggtacctaatgatttttatcaaaatcattaagttaaggtagatacacatcttgtcatatgatcaaatggtttcgccaaaaatcaataatcagacaacaagatgtgcgaactcgatattttacacgactctctttaccaattctaccacaacgtggtttgcaggagtcaggcaactatggatgaacgaaatagacagatcgctgagataggtgcctcactgattaagcattggtaactgtcagaccaagtttactcatatatactttagattgatttaaaacttcatttttaatttaaaaggatctaggtgaagatcctttttgataatctcatgaccaaaatcccttaacgtgagttttcgttccactgagcgtcagaccccgtagaaaagatcaaaggatcttcttgagatcctttttttctgcgcgtaatctgctgcttgcaaacaaaaaaaccaccgctaccagcggtggtttgtttgccggatcaagagctaccaactctttttccgaaggtaactggcttcagcagagcgcagataccaaatactgttcttctagtgtagccgtagttaggccaccacttcaagaactctgtagcaccgcctacatacctcgctctgctaatcctgttaccagtggctgctgccagtggcgataagtcgtgtcttaccgggttggactcaagacgatagttaccggataaggcgcagcggtcgggctgaacggggggttcgtgcacacagcccagcttggagcgaacgacctacaccgaactgagatacctacagcgtgagctatgagaaagcgccacgcttcccgaagggagaaaggcggacaggtatccggtaagcggcagggtcggaacaggagagcgcacgagggagcttccagggggaaacgcctggtatctttatagtcctgtcgggtttcgccacctctgacttgagcgtcgatttttgtgatgctcgtcaggggggcggagcctatggaaaaacgccagcaacgcggcctttttacggttcctggccttttgctggccttttgctcacatgttctttcctgcgttatcccctgattctgtggataaccgtattaccgcctttgagtgagctgataccgctcgccgcagccgaacgaccgagcgcagcgagtcagtgagcgaggaagcggaagagcgcctgatgcggtattttctccttacgcatctgtgcggtatttcacaccgcatatggtgcactctcagtacaatctgctctgatgccgcatagttaagccagtatacactccgctatcgctacgtgactgggtcatggctgcgccccgacacccgccaacacccgctgacgcgccctgacgggcttgtctgctcccggcatccgcttacagacaagctgtgaccgtctccgggagctgcatgtgtcagaggttttcaccgtcatcaccgaaacgcgcgaggcagcctaagaaaaaaaagcccgctcattaggcgggctagcgacgtctaatacgactcactat

SEQ ID NO: 5 - DNA, 2284 bp, synthetic construct
  misc_feature 1..2284: note = P1140-K-backbone
  source 1..2284: mol_type = other DNA
gaaaaactcatcgagcatcaaatgaaactgcaatttattcatatcaggattatcaataccatatttttgaaaaagccgtttctgtaatgaaggagaaaactcaccgaggcagttccataggatggcaagatcctggtatcggtctgcgattccgactcgtccaacatcaatacaacctatcaatttcccctcgtcaaaaataaggttatcaagtgagaaatcaccatgagtgacgactgaatccggtgagaatggcaaaagtttgtgcatttctttccagacttgttcaacaggccagccattacgctcgtcatcaaaatcactcgcatcaaccaaaccgttattcattcgtgattgcgcctgagcgagacgaaatacgcgatcgctgttaaaaggacaattacaaacaggaatcgaatgtaaccggcgcaggaacactgccagcgcatcaacaatattttcacctgaatcaggatattcttctaatacctggaaggctgttttcccagggatcgcagtggtgagtaaccaagcatcatcaggagtacggataaaatgcttgatggtcggaagaggcataaattccgtcagccagtttagtctgaccatctcatctgtaacatcattggcaacgctacctttgccatgtttcagaaacaactctggcgcatcgggcttcccatacaatcggtagattgtcgcacctgattgcccgacattatcgcgagcccatttatacccatataaatcagcatccatgttggaatttaatcgcggcctagagcaagacgtttcccgttgaatatggctcataacaccccttgtattactgtttatgtaagcagacagttttattgttcatgatgatatatttttatcttgtgcaatgtaacatcagagattttgagacacaacgtggtttgcaggagtcaggcaactatggatgaacgaaatagacagatcgctgagataggtgcctcactgattaagcattggtaactgtcagaccaagtttactcatatatactttagattgatttaaaacttcatttttaatttaaaaggatctaggtgaagatcctttttgataatctcatgaccaaaatcccttaacgtgagttttcgttccactgagcgtcagaccccgtagaaaagatcaaaggatcttcttgagatcctttttttctgcgcgtaatctgctgcttgcaaacaaaaaaaccaccgctaccagcggtggtttgtttgccggatcaagagctaccaactctttttccgaaggtaactggcttcagcagagcgcagataccaaatactgttcttctagtgtagccgtagttaggccaccacttcaagaactctgtagcaccgcctacatacctcgctctgctaatcctgttaccagtggctgctgccagtggcgataagtcgtgtcttaccgggttggactcaagacgatagttaccggataaggcgcagcggtcgggctgaacggggggttcgtgcacacagcccagcttggagcgaacgacctacaccgaactgagatacctacagcgtgagctatgagaaagcgccacgcttcccgaagggagaaaggcggacaggtatccggtaagcggcagggtcggaacaggagagcgcacgagggagcttccagggggaaacgcctggtatctttatagtcctgtcgggtttcgccacctctgacttgagcgtcgatttttgtgatgctcgtcaggggggcggagcctatggaaaaacgccagcaacgcggcctttttacggttcctggccttttgctggccttttgctcacatgttctttcctgcgttatcccctgattctgtggataaccgtattaccgcctttgagtgagctgataccgctcgccgcagccgaacgaccgagcgcagcgagtcagtgagcgaggaagcggaagagcgcctgatgcggtattttctccttacgcatctgtgcggtatttcacaccgcatatggtgcactctcagtacaatctgctctgatgccgcatagttaagccagtatacactccgctatcgctacgtgactgggtcatggctgcgccccgacacccgccaacacccgctgacgcgccctgacgggcttgtctgctcccggcatccgcttacagacaagctgtgaccgtctccgggagctgcatgtgtcagaggttttcaccgtcatcaccgaaacgcgcgaggcagcctaagaaaaaaaagcccgctcattaggcgggctagcgacgtctaatacgactcactat

SEQ ID NO: 6 - DNA, 1015 bp, synthetic construct
  misc_feature 1..1015: note = pUC origin
  source 1..1015: mol_type = other DNA
ggagtcaggcaactatggatgaacgaaatagacagatcgctgagataggtgcctcactgattaagcattggtaactgtcagaccaagtttactcatatatactttagattgatttaaaacttcatttttaatttaaaaggatctaggtgaagatcctttttgataatctcatgaccaaaatcccttaacgtgagttttcgttccactgagcgtcagaccccgtagaaaagatcaaaggatcttcttgagatcctttttttctgcgcgtaatctgctgcttgcaaacaaaaaaaccaccgctaccagcggtggtttgtttgccggatcaagagctaccaactctttttccgaaggtaactggcttcagcagagcgcagataccaaatactgttcttctagtgtagccgtagttaggccaccacttcaagaactctgtagcaccgcctacatacctcgctctgctaatcctgttaccagtggctgctgccagtggcgataagtcgtgtcttaccgggttggactcaagacgatagttaccggataaggcgcagcggtcgggctgaacggggggttcgtgcacacagcccagcttggagcgaacgacctacaccgaactgagatacctacagcgtgagctatgagaaagcgccacgcttcccgaagggagaaaggcggacaggtatccggtaagcggcagggtcggaacaggagagcgcacgagggagcttccagggggaaacgcctggtatctttatagtcctgtcgggtttcgccacctctgacttgagcgtcgatttttgtgatgctcgtcaggggggcggagcctatggaaaaacgccagcaacgcggcctttttacggttcctggccttttgctggccttttgctcacatgttctttcctgcgttatcccctgattctgtggataaccgtattaccgcctttgagtgagctgataccgctcgccgcagccgaacgaccgagcgcagcgagtcagtgagcgaggaagcggaaga

SEQ ID NO: 7 - DNA, 589 bp, synthetic construct
  misc_feature 1..589: note = pBR322 origin
  source 1..589: mol_type = other DNA
ttttccataggctccgcccccctgacgagcatcacaaaaatcgacgctcaagtcagaggtggcgaaacccgacaggactataaagataccaggcgtttccccctggaagctccctcgtgcgctctcctgttccgaccctgccgcttaccggatacctgtccgcctttctcccttcgggaagcgtggcgctttctcatagctcacgctgtaggtatctcagttcggtgtaggtcgttcgctccaagctgggctgtgtgcacgaaccccccgttcagcccgaccgctgcgccttatccggtaactatcgtcttgagtccaacccggtaagacacgacttatcgccactggcagcagccactggtaacaggattagcagagcgaggtatgtaggcggtgctacagagttcttgaagtggtggcctaactacggctacactagaaggacagtatttggtatctgcgctctgctgaagccagttaccttcggaaaaagagttggtagctcttgatccggcaaacaaaccaccgctggtagcggtggtttttttgtttgcaagcagcagattacgcgcagaaaaaaaggatctca

SEQ ID NO: 8 - DNA, 582 bp, synthetic construct
  misc_feature 1..582: note = pMB1 origin
  source 1..582: mol_type = other DNA
gcgttgctggcgtttttccataggctccgcccccctgacgagcatcacaaaaatcgacgctcaagtcagaggtggcgaaacccgacaggactataaagataccaggcgtttccccctggaagctccctcgtgcgctctcctgttccgaccctgccgcttaccggatacctgtccgcctttctcccttcgggaagcgtggcgctttctcatagctcacgctgtaggtatctcagttcggtgtaggtcgttcgctccaagctgggctgtgtgcacgaaccccccgttcagcccgaccgctgcgccttatccggtaactatcgtcttgagtccaacccggtaagacacgacttatcgccactggcagcagccactggtaacaggattagcagagcgaggtatgtaggcggtgctacagagttcttgaagtggtggcctaactacggctacactagaaggacagtatttggtatctgcgctctgctgaagccagttccttcggaaaaagagttggtagctcttgatccggcaaacaaaccaccgctggtagcggtggtttttttgtttgcaagcagcagattacgc

SEQ ID NO: 9 - DNA, 602 bp, synthetic construct
  misc_feature 1..602: note = ColE1 origin
  source 1..602: mol_type = other DNA
aggatcttcttgagatcctttttttctgcgcgtaatctgctgcttgcaaacaaaaaaaccaccgctaccaacggtggtttgtttgccggatcaagagctaccaactctttttccgaaggtaactggcttcagcagagcgcagataccaaatactgtccttctagtgtagccgtagtcgggccactacttcaagaactctgtagcaccgtttgtgccatcatcgctctgctaatccggttaccagtggctgctgccagtggcgttaaggcgtgccttaccgggttggactcaagacgatagttaccggataaggcgcagcggtcgggctgaacggggggttcgtgcacacagcccagcttggagcgaacgacctacaccgaactgagataccaacagcgtgagctatgagaaagcgccacgcttcccgaagggagaaaggcggacaggtatccggtaagcggcagggtcggaacaggagagcgcacgagggagcttccagggggaaacgcctggtatctttatagtcctgtcgggtttcgccacctctgacttgagcgtctatttttgtgatgctcgtcaggggggcggagcctatggaaaaa

SEQ ID NO: 10 - DNA, 282 bp, synthetic construct
  misc_feature 1..282: note = R6K_gamma origin
  source 1..282: mol_type = other DNA
aagctttaaaagccttatatattcttttttttcttataaaacttaaaaccttagaggctatttaagttgctgatttatattaattttattgttcaaacatgagagcttagtacgtgaaacatgagagcttagtacgttagccatgagagcttagtacgttagccatgagggtttagttcgttaaacatgagagcttagtacgttaaacatgagagcttagtacgtgaaacatgagagcttagtacgtactatcaacaggttgaactgctgatcttcagatct

SEQ ID NO: 11 - DNA, 532 bp, synthetic construct
  misc_feature 1..532: note = R6K_beta origin
  source 1..532: mol_type = other DNA
agatctatggatgttgagaatgtagtatggttatactgcgatgcaggatagggcaaacgccgtaaaatgacgtctttgacgttatttttcagcgcttgcccggtgacctacagtcggttcttgttgggagattttatgaagtttatagtaaaggattttatcagtgataaatatgcaaaggctattaacattttaaatgataaccttaaagaaaactactatgttttttatggtgtaaggttaagtgaaattctttttcctgcaagtgattatggtacagatgatttttttaaggagtttgaggaaataaacaacgttaccttgctttagttgtttttgaaataaatgaacgtgaacctgtgattgtaattggttttgatgaaataaatggtgcgattcttatagagaaatccggtataaaggttttagtaatcgataatctatcggcgttgctgaccaatgaaacattgggtgtcttcttcaagtaacagatctagctgaaaatcgtcatcaaaactgtgcaccttatctg

SEQ ID NO: 12 - DNA, 639 bp, synthetic construct
  misc_feature 1..639: note = R6K alpha origin
  source 1..639: mol_type = other DNA
tcttacttctttgcgtagctgttaaatacagcgttgttttgataaaatcatcattatcatcgataatgctttcttcaatttttttatccttactctttaataaagcacttgctaataacttcataccttttgcaactgtcaaatttggttcatcagggtaaatgcttttaaggcatactaacaaataatcatggtcttcatcttcaactctaaactgaatttttttcatcataactcccaacaagaaccgactgtaggtcaccgggcaaacgctgaaaaataacgtcgaatgacgtcattttgcggcgtttgccctatcctgcatcgcagtagaaaatgccacaactgaaattgtgcttcagtatgtacagaaatgcaaaatctgagggatttcgtagctgaaagatcgccagtcttcgaccgtaaggataggagttgctgtaagacctgtgcggggcgttcgcttcgcgaacgggtctggcagggggcacaagcgctgtgctgtgatatatgcaaaagaagccacccacgaacgggagggcttcggcgaatcgactatagtgatctatttacccggctgattgtcgccttctagccctcgcgggcatcatgcaaccagtgcctgaatttagttatatg

SEQ ID NO: 13 - DNA, 914 bp, synthetic construct
  misc_feature 1..914: note = p15A origin
  source 1..914: mol_type = other DNA
gcgctagcggagtgtatactggcttactatgttggcactgatgagggtgtcagtgaagtgcttcatgtggcaggagaaaaaaggctgcaccggtgcgtcagcagaatatgtgatacaggatatattccgcttcctcgctcactgactcgctacgctcggtcgttcgactgcggcgagcggaaatggcttacgaacggggcggagatttcctggaagatgccaggaagatacttaacagggaagtgagagggccgcggcaaagccgtttttccataggctccgcccccctgacaagcatcacgaaatctgacgctcaaatcagtggtggcgaaacccgacaggactataaagataccaggcgtttccccctggcggctccctcgtgcgctctcctgttcctgcctttcggtttaccggtgtcattccgctgttatggccgcgtttgtctcattccacgcctgacactcagttccgggtaggcagttcgctccaagctggactgtatgcacgaaccccccgttcagtccgaccgctgcgccttatccggtaactatcgtcttgagtccaacccggaaagacatgcaaaagcaccactggcagcagccactggtaattgatttagaggagttagtcttgaagtcatgcgccggttaaggctaaactgaaaggacaagttttggtgactgcgctcctccaagccagttacctcggttcaaagagttggtagctcagagaaccttcgaaaaaccgccctgcaaggcggttttttcgttttcagagcaagagattacgcgcagaccaaaacgatctcaagaagatcatcttattaatcagataaaatatttctagttttcagtgcaatttatctcttcaaatgtagcacctgaagtcagccccatacgatataagttgta

SEQ ID NO: 14 - DNA, 300 bp, synthetic construct
  misc_feature 1..300: note = pSC101 origin
  source 1..300: mol_type = other DNA
gcggaactgactaaagtagtgagttatacacagggctgggatctattctttttatctttttttattctttctttattctataaattataaccacttgaatataaacaaaaaaaacacacaaaggtctagcggaatttacagagggtctagcagaatttacaagttttccagcaaaggtctagcagaatttacagatacccacaactcaaaggaaaaggactagtaattatcattgactagcccatctcaattggtatagtgattaaaatcacctagaccaattgagatgtatgtctgaat

SEQ ID NO: 15 - DNA, 307 bp, synthetic construct
  misc_feature 1..307: note = F1 phagemid origin
  source 1..307: mol_type = other DNA
ttgttccagtttggaacaagagtccactattaaagaacgtggactccaacgtcaaagggcgaaaaaccgtctatcagggcgatggcccactacgtgaaccatcaccctaatcaagttttttggggtcgaggtgccgtaaagcactaaatcggaaccctaaagggagcccccgatttagagcttgacggggaaagccggcgaacgtggcgagaaaggaagggaagaaagcgaaaggagcgggcgctagggcgctggcaagtgtagcggtcacgctgcgcgtaaccaccacacccgccgcgcttaatgc

SEQ ID NO: 16 - DNA, 24 bp, synthetic construct
  misc_feature 1..24: note = histone stem-loop
  source 1..24: mol_type = other DNA
caaaggctcttttcagagccacca

SEQ ID NO: 17 - RNA, 24 nt, synthetic construct
  misc_feature 1..24: note = histone stem loop
  source 1..24: mol_type = other RNA
caaaggctcttttcagagccacca